European Patent Application EP 4 484 551 A1, published January 1, 2025. Title: USE OF BCG GENE BCG_1820 IN PREPARING TUBERCULOSIS VACCINE RECOMBINANT BCG. Applicant: SHANGHAI PULMONARY HOSPITAL. The sequence listing filed with the application follows.

SEQUENCE LISTING (2 sequences)

SEQ ID NO: 1 - protein, 99 aa, Mycobacterium bovis
MSFVTTQPEALAAAAGSLQGIGSALNAQNAAAATPTTGVVPAAADEVSALTAAQFAAHAQIYQAVSAQAAAIHEMFVNTLQMSSGSYAATEAANAAAAG

SEQ ID NO: 2 - DNA, 20 bp, Artificial Sequence
atcggctccgcattgaacgc